European Patent Application EP 4 803 151 A2, published September 9, 2026. Title: ANTI-DLL3 ANTIBODIES AND USES THEREOF. Applicant: Concept to Medicine Biotech Co., Ltd. The sequence listing filed with the application follows.

SEQUENCE LISTING (125 sequences)

SEQ ID NO: 1 - protein, 115 aa, synthetic construct
QVQLQQSGAELVRPGASVKLSCKALGYTFTDSEIHWVKQTPVHGLEWIGAIHPRNGGTAYNQKFRGKATLSADRSSNTAYMELSSLTSEDSAVYYCSRGYFLDYWGQGTSVTVSS

SEQ ID NO: 2 - protein, 113 aa, synthetic construct
DIVMTQSPSSLTMSVGQKVTMSCKSSQSLLNSDNQKNYLAWYQQRPGQSPKLLLYFASTRESGVPDRFIGSGSGTDFTLTISSVQAEDLADYFCQHHYDTPPTFGGGTKLEIK

SEQ ID NO: 3 - protein, 112 aa, synthetic construct
QVQLQQSGPELVKPGASVKISCRASGYTFTDHHLNWVKQRPGQGLEWIGWIFPGSGSDYYNERFKDKATLTVDKSSSTAYMLLSSLTSEDSAVYFCERWDYWGQGTTLTVSS

SEQ ID NO: 4 - protein, 106 aa, synthetic construct
QIVLTQSPTIMSASPGEKVTMTCSASSSISYMHWYQQKPGTSPKRWIYDTSTLASGVPARFSGGGSGTSYSLTISSMEAEDAATYYCHQRSSYPLTFGAGTKLELK

SEQ ID NO: 5 - protein, 116 aa, synthetic construct
EVNLEESGGGLVQPGGSMKLSCVVSGFTFSNYWMSWVRQSPEKGLEWVAEIRLKSDNYATHYAESVKGKFTISRDDSKSRLYLQMNSLRPEDTGIYYCTSNRFAYWGQGTLVTVSA

SEQ ID NO: 6 - protein, 107 aa, synthetic construct
NIVMTQSPKSVSMSVGERVTLSCKASENVGTYVYWYQQKPEQSPKMMIYGASNRYTGVPDRFTGSGSATDFTLTIRSVQAEDLADYHCGQSYSYPFTFGSGTKLEIK

SEQ ID NO: 7 - protein, 121 aa, synthetic construct
EVQLQQSGPELIKPGTSVKMSCKASGYTFTTYLMHWVKQKPGQGLEWIGYINPYNDVTEYHEKFKDKATLTSDKSSSTAYMELSSLTSEDSAVYYCARLGGYGPGWYLDVWGAGTTVTVSS

SEQ ID NO: 8 - protein, 107 aa, synthetic construct
DIQMTQSPASLSASVGETVTITCRASGSIHNYLAWYLHKQGKSPQLLVYNAKTLADGVPSRFSGSGSGTQYSLKINSLQPEDFGSYYCHHFWSTPWTFGGGTKLEIK

SEQ ID NO: 9 - protein, 118 aa, synthetic construct
EVQLQQSGPELVKPGASVKISCKASGYTFTDFYMNWVKQTHGKSLEWIGDANPNNGGTTHNPRFKGQATLTVDKSSNTAYMELRSLTSEDSAVYYCARGGLPGDFDYWGQGTTLTVSS

SEQ ID NO: 10 - protein, 107 aa, synthetic construct
DIQMTQSSSSFSVSLGDRVTITCKASEDIYNRLAWYQQKPGNAPRLLISGVTSLETGVPSRFSGSGSGKDYTLSITSLQTEDVATYYCQQYWSFPWTFGGGTKLEIK

SEQ ID NO: 11 - protein, 122 aa, synthetic construct
EVQLQQSGPELLKPGASVKISCKASGYTFTDYTMHWVKQSHGRSLEWIGGIHPNYGGTSYNEKFKDKATLTVDKSSSTAYMEFRSLTSEDSAVYYCARWGYYGGSYWYFDVWGTGTTVTVSS

SEQ ID NO: 12 - protein, 107 aa, synthetic construct
DIQMTQSPASLSVSVGETVTITCRASENIYSNLAWYQQKQGKSPQLLVYAATNLADGVPSRFSGSGSGTQYSLKINSLQSEDFGSYYCQHFWGTPYTFGGGTKLEIK

SEQ ID NO: 13 - protein, 5 aa, synthetic construct
DSEIH

SEQ ID NO: 14 - protein, 17 aa, synthetic construct
AIHPRNGGTAYNQKFRG

SEQ ID NO: 15 - protein, 6 aa, synthetic construct
GYFLDY

SEQ ID NO: 16 - protein, 17 aa, synthetic construct
KSSQSLLNSDNQKNYLA

SEQ ID NO: 17 - protein, 7 aa, synthetic construct
FASTRES

SEQ ID NO: 18 - protein, 9 aa, synthetic construct
QHHYDTPPT

SEQ ID NO: 19 - protein, 5 aa, synthetic construct
DHHLN

SEQ ID NO: 20 - protein, 17 aa, synthetic construct
WIFPGSGSDYYNERFKD

SEQ ID NO: 21 - skipped

SEQ ID NO: 22 - protein, 10 aa, synthetic construct
SASSSISYMH

SEQ ID NO: 23 - protein, 7 aa, synthetic construct
DTSTLAS

SEQ ID NO: 24 - protein, 9 aa, synthetic construct
HQRSSYPLT

SEQ ID NO: 25 - protein, 5 aa, synthetic construct
NYWMS

SEQ ID NO: 26 - protein, 19 aa, synthetic construct
EIRLKSDNYATHYAESVKG

SEQ ID NO: 27 - protein, 5 aa, synthetic construct
NRFAY

SEQ ID NO: 28 - protein, 11 aa, synthetic construct
KASENVGTYVY

SEQ ID NO: 29 - protein, 7 aa, synthetic construct
GASNRYT

SEQ ID NO: 30 - protein, 9 aa, synthetic construct
GQSYSYPFT

SEQ ID NO: 31 - protein, 5 aa, synthetic construct
TYLMH

SEQ ID NO: 32 - protein, 17 aa, synthetic construct
YINPYNDVTEYHEKFKD

SEQ ID NO: 33 - protein, 12 aa, synthetic construct
LGGYGPGWYLDV

SEQ ID NO: 34 - protein, 11 aa, synthetic construct
RASGSIHNYLA

SEQ ID NO: 35 - protein, 7 aa, synthetic construct
NAKTLAD

SEQ ID NO: 36 - protein, 9 aa, synthetic construct
HHFWSTPWT

SEQ ID NO: 37 - protein, 5 aa, synthetic construct
DFYMN

SEQ ID NO: 38 - protein, 17 aa, synthetic construct
DANPNNGGTTHNPRFKG

SEQ ID NO: 39 - protein, 9 aa, synthetic construct
GGLPGDFDY

SEQ ID NO: 40 - protein, 11 aa, synthetic construct
KASEDIYNRLA

SEQ ID NO: 41 - protein, 7 aa, synthetic construct
GVTSLET

SEQ ID NO: 42 - protein, 9 aa, synthetic construct
QQYWSFPWT

SEQ ID NO: 43 - protein, 5 aa, synthetic construct
DYTMH

SEQ ID NO: 44 - protein, 17 aa, synthetic construct
GIHPNYGGTSYNEKFKD

SEQ ID NO: 45 - protein, 13 aa, synthetic construct
WGYYGGSYWYFDV

SEQ ID NO: 46 - protein, 11 aa, synthetic construct
RASENIYSNLA

SEQ ID NO: 47 - protein, 7 aa, synthetic construct
AATNLAD

SEQ ID NO: 48 - protein, 9 aa, synthetic construct
QHFWGTPYT

SEQ ID NO: 49 - protein, 445 aa, synthetic construct
QVQLQQSGAELVRPGASVKLSCKALGYTFTDSEIHWVKQTPVHGLEWIGAIHPRNGGTAYNQKFRGKATLSADRSSNTAYMELSSLTSEDSAVYYCSRGYFLDYWGQGTSVTVSSASTKGPSVFPLAPSSKSTSGGTAALGCLVKDYFPEPVTVSWNSGALTSGVHTFPAVLQSSGLYSLSSVVTVPSSSLGTQTYICNVNHKPSNTKVDKKVEPKSCDKTHTCPPCPAPELLGGPSVFLFPPKPKDTLMISRTPEVTCVVVDVSHEDPEVKFNWYVDGVEVHNAKTKPREEQYNSTYRVVSVLTVLHQDWLNGKEYKCKVSNKALPAPIEKTISKAKGQPREPQVYTLPPSREEMTKNQVSLTCLVKGFYPSDIAVEWESNGQPENNYKTTPPVLDSDGSFFLYSKLTVDKSRWQQGNVFSCSVMHEALHNHYTQKSLSLSPGK

SEQ ID NO: 50 - protein, 220 aa, synthetic construct
DIVMTQSPSSLTMSVGQKVTMSCKSSQSLLNSDNQKNYLAWYQQRPGQSPKLLLYFASTRESGVPDRFIGSGSGTDFTLTISSVQAEDLADYFCQHHYDTPPTFGGGTKLEIKRTVAAPSVFIFPPSDEQLKSGTASVVCLLNNFYPREAKVQWKVDNALQSGNSQESVTEQDSKDSTYSLSSTLTLSKADYEKHKVYACEVTHQGLSSPVTKSFNRGEC

SEQ ID NO: 51 - protein, 442 aa, synthetic construct
QVQLQQSGPELVKPGASVKISCRASGYTFTDHHLNWVKQRPGQGLEWIGWIFPGSGSDYYNERFKDKATLTVDKSSSTAYMLLSSLTSEDSAVYFCERWDYWGQGTTLTVSSASTKGPSVFPLAPSSKSTSGGTAALGCLVKDYFPEPVTVSWNSGALTSGVHTFPAVLQSSGLYSLSSVVTVPSSSLGTQTYICNVNHKPSNTKVDKKVEPKSCDKTHTCPPCPAPELLGGPSVFLFPPKPKDTLMISRTPEVTCVVVDVSHEDPEVKFNWYVDGVEVHNAKTKPREEQYNSTYRVVSVLTVLHQDWLNGKEYKCKVSNKALPAPIEKTISKAKGQPREPQVYTLPPSREEMTKNQVSLTCLVKGFYPSDIAVEWESNGQPENNYKTTPPVLDSDGSFFLYSKLTVDKSRWQQGNVFSCSVMHEALHNHYTQKSLSLSPGK

SEQ ID NO: 52 - protein, 213 aa, synthetic construct
QIVLTQSPTIMSASPGEKVTMTCSASSSISYMHWYQQKPGTSPKRWIYDTSTLASGVPARFSGGGSGTSYSLTISSMEAEDAATYYCHQRSSYPLTFGAGTKLELKRTVAAPSVFIFPPSDEQLKSGTASVVCLLNNFYPREAKVQWKVDNALQSGNSQESVTEQDSKDSTYSLSSTLTLSKADYEKHKVYACEVTHQGLSSPVTKSFNRGEC

SEQ ID NO: 53 - protein, 446 aa, synthetic construct
EVNLEESGGGLVQPGGSMKLSCVVSGFTFSNYWMSWVRQSPEKGLEWVAEIRLKSDNYATHYAESVKGKFTISRDDSKSRLYLQMNSLRPEDTGIYYCTSNRFAYWGQGTLVTVSAASTKGPSVFPLAPSSKSTSGGTAALGCLVKDYFPEPVTVSWNSGALTSGVHTFPAVLQSSGLYSLSSVVTVPSSSLGTQTYICNVNHKPSNTKVDKKVEPKSCDKTHTCPPCPAPELLGGPSVFLFPPKPKDTLMISRTPEVTCVVVDVSHEDPEVKFNWYVDGVEVHNAKTKPREEQYNSTYRVVSVLTVLHQDWLNGKEYKCKVSNKALPAPIEKTISKAKGQPREPQVYTLPPSREEMTKNQVSLTCLVKGFYPSDIAVEWESNGQPENNYKTTPPVLDSDGSFFLYSKLTVDKSRWQQGNVFSCSVMHEALHNHYTQKSLSLSPGK

SEQ ID NO: 54 - protein, 214 aa, synthetic construct
NIVMTQSPKSVSMSVGERVTLSCKASENVGTYVYWYQQKPEQSPKMMIYGASNRYTGVPDRFTGSGSATDFTLTIRSVQAEDLADYHCGQSYSYPFTFGSGTKLEIKRTVAAPSVFIFPPSDEQLKSGTASVVCLLNNFYPREAKVQWKVDNALQSGNSQESVTEQDSKDSTYSLSSTLTLSKADYEKHKVYACEVTHQGLSSPVTKSFNRGEC

SEQ ID NO: 55 - protein, 451 aa, synthetic construct
EVQLQQSGPELIKPGTSVKMSCKASGYTFTTYLMHWVKQKPGQGLEWIGYINPYNDVTEYHEKFKDKATLTSDKSSSTAYMELSSLTSEDSAVYYCARLGGYGPGWYLDVWGAGTTVTVSSASTKGPSVFPLAPSSKSTSGGTAALGCLVKDYFPEPVTVSWNSGALTSGVHTFPAVLQSSGLYSLSSVVTVPSSSLGTQTYICNVNHKPSNTKVDKKVEPKSCDKTHTCPPCPAPELLGGPSVFLFPPKPKDTLMISRTPEVTCVVVDVSHEDPEVKFNWYVDGVEVHNAKTKPREEQYNSTYRVVSVLTVLHQDWLNGKEYKCKVSNKALPAPIEKTISKAKGQPREPQVYTLPPSREEMTKNQVSLTCLVKGFYPSDIAVEWESNGQPENNYKTTPPVLDSDGSFFLYSKLTVDKSRWQQGNVFSCSVMHEALHNHYTQKSLSLSPGK

SEQ ID NO: 56 - protein, 214 aa, synthetic construct
DIQMTQSPASLSASVGETVTITCRASGSIHNYLAWYLHKQGKSPQLLVYNAKTLADGVPSRFSGSGSGTQYSLKINSLQPEDFGSYYCHHFWSTPWTFGGGTKLEIKRTVAAPSVFIFPPSDEQLKSGTASVVCLLNNFYPREAKVQWKVDNALQSGNSQESVTEQDSKDSTYSLSSTLTLSKADYEKHKVYACEVTHQGLSSPVTKSFNRGEC

SEQ ID NO: 57 - protein, 448 aa, synthetic construct
EVQLQQSGPELVKPGASVKISCKASGYTFTDFYMNWVKQTHGKSLEWIGDANPNNGGTTHNPRFKGQATLTVDKSSNTAYMELRSLTSEDSAVYYCARGGLPGDFDYWGQGTTLTVSSASTKGPSVFPLAPSSKSTSGGTAALGCLVKDYFPEPVTVSWNSGALTSGVHTFPAVLQSSGLYSLSSVVTVPSSSLGTQTYICNVNHKPSNTKVDKKVEPKSCDKTHTCPPCPAPELLGGPSVFLFPPKPKDTLMISRTPEVTCVVVDVSHEDPEVKFNWYVDGVEVHNAKTKPREEQYNSTYRVVSVLTVLHQDWLNGKEYKCKVSNKALPAPIEKTISKAKGQPREPQVYTLPPSREEMTKNQVSLTCLVKGFYPSDIAVEWESNGQPENNYKTTPPVLDSDGSFFLYSKLTVDKSRWQQGNVFSCSVMHEALHNHYTQKSLSLSPGK

SEQ ID NO: 58 - protein, 214 aa, synthetic construct
DIQMTQSSSSFSVSLGDRVTITCKASEDIYNRLAWYQQKPGNAPRLLISGVTSLETGVPSRFSGSGSGKDYTLSITSLQTEDVATYYCQQYWSFPWTFGGGTKLEIKRTVAAPSVFIFPPSDEQLKSGTASVVCLLNNFYPREAKVQWKVDNALQSGNSQESVTEQDSKDSTYSLSSTLTLSKADYEKHKVYACEVTHQGLSSPVTKSFNRGEC

SEQ ID NO: 59 - protein, 452 aa, synthetic construct
EVQLQQSGPELLKPGASVKISCKASGYTFTDYTMHWVKQSHGRSLEWIGGIHPNYGGTSYNEKFKDKATLTVDKSSSTAYMEFRSLTSEDSAVYYCARWGYYGGSYWYFDVWGTGTTVTVSSASTKGPSVFPLAPSSKSTSGGTAALGCLVKDYFPEPVTVSWNSGALTSGVHTFPAVLQSSGLYSLSSVVTVPSSSLGTQTYICNVNHKPSNTKVDKKVEPKSCDKTHTCPPCPAPELLGGPSVFLFPPKPKDTLMISRTPEVTCVVVDVSHEDPEVKFNWYVDGVEVHNAKTKPREEQYNSTYRVVSVLTVLHQDWLNGKEYKCKVSNKALPAPIEKTISKAKGQPREPQVYTLPPSREEMTKNQVSLTCLVKGFYPSDIAVEWESNGQPENNYKTTPPVLDSDGSFFLYSKLTVDKSRWQQGNVFSCSVMHEALHNHYTQKSLSLSPGK

SEQ ID NO: 60 - protein, 214 aa, synthetic construct
DIQMTQSPASLSVSVGETVTITCRASENIYSNLAWYQQKQGKSPQLLVYAATNLADGVPSRFSGSGSGTQYSLKINSLQSEDFGSYYCQHFWGTPYTFGGGTKLEIKRTVAAPSVFIFPPSDEQLKSGTASVVCLLNNFYPREAKVQWKVDNALQSGNSQESVTEQDSKDSTYSLSSTLTLSKADYEKHKVYACEVTHQGLSSPVTKSFNRGEC

SEQ ID NO: 61 - protein, 98 aa, synthetic construct
QVQLVQSGAEVKKPGASVKVSCKASGYTFTSYGISWVRQAPGQGLEWMGWISAYNGNTNYAQKLQGRVTMTTDTSTSTAYMELRSLRSDDTAVYYCAR

SEQ ID NO: 62 - protein, 98 aa, synthetic construct
QVQLVQSGAEVKKPGASVKVSCKASGYTFTSYAMHWVRQAPGQRLEWMGWINAGNGNTKYSQKFQGRVTITRDTSASTAYMELSSLRSEDTAVYYCAR

SEQ ID NO: 63 - protein, 95 aa, synthetic construct
DIQMTQSPSSVSASVGDRVTITCRASQGISSWLAWYQQKPGKAPKLLIYAASSLQSGVPSRFSGSGSGTDFTLTISSLQPEDFATYYCQQANSFP

SEQ ID NO: 64 - protein, 95 aa, synthetic construct
DIQMTQSPSSLSASVGDRVTITCQASQDISNYLNWYQQKPGKAPKLLIYDASNLETGVPSRFSGSGSGTDFTFTISSLQPEDIATYYCQQYDNLP

SEQ ID NO: 65 - protein, 118 aa, synthetic construct
QVQLVQSGAEVKKPGASVKVSCKASGYTFTDFYMNWVRQAPGQGLEWMGDANPNNGGTTHNPRFKGRVTMTTDTSTSTAYMELRSLRSDDTAVYYCARGGLPGDFDYWGQGTTVTVSS

SEQ ID NO: 66 - protein, 118 aa, synthetic construct
QVQLVQSGAEVKKPGASVKVSCKASGYTFTDFYMNWVRQAPGQGLEWIGDANPNNGGTTHNPRFKGRATMTTDTSTSTAYMELRSLRSDDTAVYYCARGGLPGDFDYWGQGTTVTVSS

SEQ ID NO: 67 - protein, 118 aa, synthetic construct
QVQLVQSGAEVKKPGASVKVSCKASGYTFTDFYMNWVRQAPGQGLEWIGDANPNNGGTTHNPRFKGRATLTVDTSTSTAYMELRSLRSDDTAVYYCARGGLPGDFDYWGQGTTVTVSS

SEQ ID NO: 68 - protein, 118 aa, synthetic construct
QVQLVQSGAEVKKPGASVKVSCKASGYTFTDFYMNWVRQAPGQGLEWIGDANPNNGGTTHNPRFKGQATLTVDKSTSTAYMELRSLRSDDTAVYYCARGGLPGDFDYWGQGTTVTVSS

SEQ ID NO: 69 - protein, 118 aa, synthetic construct
QVQLVQSGAEVKKPGASVKVSCKASGYTFTDFYMNWVKQAPGQGLEWIGDANPNNGGTTHNPRFKGRATLTVDKSASTAYMELRSLRSEDTAVYYCARGGLPGDFDYWGQGTTVTVSS

SEQ ID NO: 70 - protein, 107 aa, synthetic construct
DIQMTQSPSSVSASVGDRVTITCKASEDIYNRLAWYQQKPGKAPKLLIYGVTSLETGVPSRFSGSGSGTDFTLTISSLQPEDFATYYCQQYWSFPWTFGGGTKVEIK

SEQ ID NO: 71 - protein, 107 aa, synthetic construct
DIQMTQSPSSVSASVGDRVTITCKASEDIYNRLAWYQQKPGKAPKLLISGVTSLETGVPSRFSGSGSGTDFTLTISSLQPEDFATYYCQQYWSFPWTFGGGTKVEIK

SEQ ID NO: 72 - protein, 107 aa, synthetic construct
DIQMTQSPSSVSASVGDRVTITCKASEDIYNRLAWYQQKPGKAPKLLISGVTSLETGVPSRFSGSGSGKDFTLTISSLQPEDFATYYCQQYWSFPWTFGGGTKVEIK

SEQ ID NO: 73 - protein, 107 aa, synthetic construct
DIQMTQSPSSLSASVGDRVTITCKASEDIYNRLAWYQQKPGKAPKLLISGVTSLETGVPSRFSGSGSGTDFTFTISSLQPEDIATYYCQQYWSFPWTFGGGTKVEIK

SEQ ID NO: 74 - protein, 448 aa, synthetic construct
QVQLVQSGAEVKKPGASVKVSCKASGYTFTDFYMNWVRQAPGQGLEWMGDANPNNGGTTHNPRFKGRVTMTTDTSTSTAYMELRSLRSDDTAVYYCARGGLPGDFDYWGQGTTVTVSSASTKGPSVFPLAPSSKSTSGGTAALGCLVKDYFPEPVTVSWNSGALTSGVHTFPAVLQSSGLYSLSSVVTVPSSSLGTQTYICNVNHKPSNTKVDKKVEPKSCDKTHTCPPCPAPELLGGPSVFLFPPKPKDTLMISRTPEVTCVVVDVSHEDPEVKFNWYVDGVEVHNAKTKPREEQYNSTYRVVSVLTVLHQDWLNGKEYKCKVSNKALPAPIEKTISKAKGQPREPQVYTLPPSREEMTKNQVSLTCLVKGFYPSDIAVEWESNGQPENNYKTTPPVLDSDGSFFLYSKLTVDKSRWQQGNVFSCSVMHEALHNHYTQKSLSLSPGK

SEQ ID NO: 75 - protein, 214 aa, synthetic construct
DIQMTQSPSSVSASVGDRVTITCKASEDIYNRLAWYQQKPGKAPKLLIYGVTSLETGVPSRFSGSGSGTDFTLTISSLQPEDFATYYCQQYWSFPWTFGGGTKVEIKRTVAAPSVFIFPPSDEQLKSGTASVVCLLNNFYPREAKVQWKVDNALQSGNSQESVTEQDSKDSTYSLSSTLTLSKADYEKHKVYACEVTHQGLSSPVTKSFNRGEC

SEQ ID NO: 76 - protein, 448 aa, synthetic construct
QVQLVQSGAEVKKPGASVKVSCKASGYTFTDFYMNWVRQAPGQGLEWIGDANPNNGGTTHNPRFKGRATMTTDTSTSTAYMELRSLRSDDTAVYYCARGGLPGDFDYWGQGTTVTVSSASTKGPSVFPLAPSSKSTSGGTAALGCLVKDYFPEPVTVSWNSGALTSGVHTFPAVLQSSGLYSLSSVVTVPSSSLGTQTYICNVNHKPSNTKVDKKVEPKSCDKTHTCPPCPAPELLGGPSVFLFPPKPKDTLMISRTPEVTCVVVDVSHEDPEVKFNWYVDGVEVHNAKTKPREEQYNSTYRVVSVLTVLHQDWLNGKEYKCKVSNKALPAPIEKTISKAKGQPREPQVYTLPPSREEMTKNQVSLTCLVKGFYPSDIAVEWESNGQPENNYKTTPPVLDSDGSFFLYSKLTVDKSRWQQGNVFSCSVMHEALHNHYTQKSLSLSPGK

SEQ ID NO: 77 - protein, 214 aa, synthetic construct; identical to SEQ ID NO: 75

SEQ ID NO: 78 - protein, 448 aa, synthetic construct
QVQLVQSGAEVKKPGASVKVSCKASGYTFTDFYMNWVRQAPGQGLEWIGDANPNNGGTTHNPRFKGRATLTVDTSTSTAYMELRSLRSDDTAVYYCARGGLPGDFDYWGQGTTVTVSSASTKGPSVFPLAPSSKSTSGGTAALGCLVKDYFPEPVTVSWNSGALTSGVHTFPAVLQSSGLYSLSSVVTVPSSSLGTQTYICNVNHKPSNTKVDKKVEPKSCDKTHTCPPCPAPELLGGPSVFLFPPKPKDTLMISRTPEVTCVVVDVSHEDPEVKFNWYVDGVEVHNAKTKPREEQYNSTYRVVSVLTVLHQDWLNGKEYKCKVSNKALPAPIEKTISKAKGQPREPQVYTLPPSREEMTKNQVSLTCLVKGFYPSDIAVEWESNGQPENNYKTTPPVLDSDGSFFLYSKLTVDKSRWQQGNVFSCSVMHEALHNHYTQKSLSLSPGK

SEQ ID NO: 79 - protein, 214 aa, synthetic construct; identical to SEQ ID NO: 75

SEQ ID NO: 80 - protein, 448 aa, synthetic construct
QVQLVQSGAEVKKPGASVKVSCKASGYTFTDFYMNWVRQAPGQGLEWIGDANPNNGGTTHNPRFKGQATLTVDKSTSTAYMELRSLRSDDTAVYYCARGGLPGDFDYWGQGTTVTVSSASTKGPSVFPLAPSSKSTSGGTAALGCLVKDYFPEPVTVSWNSGALTSGVHTFPAVLQSSGLYSLSSVVTVPSSSLGTQTYICNVNHKPSNTKVDKKVEPKSCDKTHTCPPCPAPELLGGPSVFLFPPKPKDTLMISRTPEVTCVVVDVSHEDPEVKFNWYVDGVEVHNAKTKPREEQYNSTYRVVSVLTVLHQDWLNGKEYKCKVSNKALPAPIEKTISKAKGQPREPQVYTLPPSREEMTKNQVSLTCLVKGFYPSDIAVEWESNGQPENNYKTTPPVLDSDGSFFLYSKLTVDKSRWQQGNVFSCSVMHEALHNHYTQKSLSLSPGK

SEQ ID NO: 81 - protein, 214 aa, synthetic construct; identical to SEQ ID NO: 75

SEQ ID NO: 82 - protein, 448 aa, synthetic construct; identical to SEQ ID NO: 74

SEQ ID NO: 83 - protein, 214 aa, synthetic construct
DIQMTQSPSSVSASVGDRVTITCKASEDIYNRLAWYQQKPGKAPKLLISGVTSLETGVPSRFSGSGSGTDFTLTISSLQPEDFATYYCQQYWSFPWTFGGGTKVEIKRTVAAPSVFIFPPSDEQLKSGTASVVCLLNNFYPREAKVQWKVDNALQSGNSQESVTEQDSKDSTYSLSSTLTLSKADYEKHKVYACEVTHQGLSSPVTKSFNRGEC

SEQ ID NO: 84 - protein, 448 aa, synthetic construct; identical to SEQ ID NO: 76

SEQ ID NO: 85 - protein, 214 aa, synthetic construct; identical to SEQ ID NO: 83

SEQ ID NO: 86 - protein, 448 aa, synthetic construct; identical to SEQ ID NO: 78

SEQ ID NO: 87 - protein, 214 aa, synthetic construct; identical to SEQ ID NO: 83

SEQ ID NO: 88 - protein, 448 aa, synthetic construct; identical to SEQ ID NO: 80

SEQ ID NO: 89 - protein, 214 aa, synthetic construct; identical to SEQ ID NO: 83

SEQ ID NO: 90 - protein, 448 aa, synthetic construct; identical to SEQ ID NO: 74

SEQ ID NO: 91 - protein, 214 aa, synthetic construct
DIQMTQSPSSVSASVGDRVTITCKASEDIYNRLAWYQQKPGKAPKLLISGVTSLETGVPSRFSGSGSGKDFTLTISSLQPEDFATYYCQQYWSFPWTFGGGTKVEIKRTVAAPSVFIFPPSDEQLKSGTASVVCLLNNFYPREAKVQWKVDNALQSGNSQESVTEQDSKDSTYSLSSTLTLSKADYEKHKVYACEVTHQGLSSPVTKSFNRGEC

SEQ ID NO: 92 - protein, 448 aa, synthetic construct; identical to SEQ ID NO: 76

SEQ ID NO: 93 - protein, 214 aa, synthetic construct; identical to SEQ ID NO: 91

SEQ ID NO: 94 - protein, 448 aa, synthetic construct; identical to SEQ ID NO: 78

SEQ ID NO: 95 - protein, 214 aa, synthetic construct; identical to SEQ ID NO: 91

SEQ ID NO: 96 - protein, 448 aa, synthetic construct; identical to SEQ ID NO: 80

SEQ ID NO: 97 - protein, 214 aa, synthetic construct; identical to SEQ ID NO: 91

SEQ ID NO: 98 - protein, 448 aa, synthetic construct; identical to SEQ ID NO: 74

SEQ ID NO: 99 - protein, 214 aa, synthetic construct
DIQMTQSPSSLSASVGDRVTITCKASEDIYNRLAWYQQKPGKAPKLLISGVTSLETGVPSRFSGSGSGTDFTFTISSLQPEDIATYYCQQYWSFPWTFGGGTKVEIKRTVAAPSVFIFPPSDEQLKSGTASVVCLLNNFYPREAKVQWKVDNALQSGNSQESVTEQDSKDSTYSLSSTLTLSKADYEKHKVYACEVTHQGLSSPVTKSFNRGEC

SEQ ID NO: 100 - protein, 448 aa, synthetic construct
QVQLVQSGAEVKKPGASVKVSCKASGYTFTDFYMNWVKQAPGQGLEWIGDANPNNGGTTHNPRFKGRATLTVDKSASTAYMELRSLRSEDTAVYYCARGGLPGDFDYWGQGTTVTVSSASTKGPSVFPLAPSSKSTSGGTAALGCLVKDYFPEPVTVSWNSGALTSGVHTFPAVLQSSGLYSLSSVVTVPSSSLGTQTYICNVNHKPSNTKVDKKVEPKSCDKTHTCPPCPAPELLGGPSVFLFPPKPKDTLMISRTPEVTCVVVDVSHEDPEVKFNWYVDGVEVHNAKTKPREEQYNSTYRVVSVLTVLHQDWLNGKEYKCKVSNKALPAPIEKTISKAKGQPREPQVYTLPPSREEMTKNQVSLTCLVKGFYPSDIAVEWESNGQPENNYKTTPPVLDSDGSFFLYSKLTVDKSRWQQGNVFSCSVMHEALHNHYTQKSLSLSPGK

SEQ ID NO: 101 - protein, 214 aa, synthetic construct; identical to SEQ ID NO: 75

SEQ ID NO: 102 - protein, 448 aa, synthetic construct; identical to SEQ ID NO: 100

SEQ ID NO: 103 - protein, 214 aa, synthetic construct; identical to SEQ ID NO: 99

SEQ ID NO: 104 - protein, 118 aa, synthetic construct
QVQLVQSGAEVKKPGASVKVSCKASGYTFTDFYMNWVKQAPGQGLEWIGDANPNAGGTTHNPRFKGRATLTVDKSASTAYMELRSLRSEDTAVYYCARGGLPGDFDYWGQGTTVTVSS

SEQ ID NO: 105 - protein, 118 aa, synthetic construct
QVQLVQSGAEVKKPGASVKVSCKASGYTFTDFYMNWVKQAPGQGLEWIGDANPNFGGTTHNPRFKGRATLTVDKSASTAYMELRSLRSEDTAVYYCARGGLPGDFDYWGQGTTVTVSS

SEQ ID NO: 106 - protein, 118 aa, synthetic construct
QVQLVQSGAEVKKPGASVKVSCKASGYTFTDFYMNWVKQAPGQGLEWIGDANPNHGGTTHNPRFKGRATLTVDKSASTAYMELRSLRSEDTAVYYCARGGLPGDFDYWGQGTTVTVSS

SEQ ID NO: 107 - protein, 118 aa, synthetic construct
QVQLVQSGAEVKKPGASVKVSCKASGYTFTDFYMNWVKQAPGQGLEWIGDANPNRGGTTHNPRFKGRATLTVDKSASTAYMELRSLRSEDTAVYYCARGGLPGDFDYWGQGTTVTVSS

SEQ ID NO: 108 - protein, 118 aa, synthetic construct
QVQLVQSGAEVKKPGASVKVSCKASGYTFTDFYMNWVKQAPGQGLEWIGDANPNVGGTTHNPRFKGRATLTVDKSASTAYMELRSLRSEDTAVYYCARGGLPGDFDYWGQGTTVTVSS

SEQ ID NO: 109 - protein, 118 aa, synthetic construct
QVQLVQSGAEVKKPGASVKVSCKASGYTFTDFYMNWVKQAPGQGLEWIGDANPNWGGTTHNPRFKGRATLTVDKSASTAYMELRSLRSEDTAVYYCARGGLPGDFDYWGQGTTVTVSS

SEQ ID NO: 110 - protein, 118 aa, synthetic construct
QVQLVQSGAEVKKPGASVKVSCKASGYTFTDFYMNWVKQAPGQGLEWIGDANPNYGGTTHNPRFKGRATLTVDKSASTAYMELRSLRSEDTAVYYCARGGLPGDFDYWGQGTTVTVSS

SEQ ID NO: 111 - protein, 17 aa, synthetic construct
DANPNAGGTTHNPRFKG

SEQ ID NO: 112 - protein, 17 aa, synthetic construct
DANPNFGGTTHNPRFKG

SEQ ID NO: 113 - protein, 17 aa, synthetic construct
DANPNHGGTTHNPRFKG

SEQ ID NO: 114 - protein, 17 aa, synthetic construct
DANPNRGGTTHNPRFKG

SEQ ID NO: 115 - protein, 17 aa, synthetic construct
DANPNVGGTTHNPRFKG

SEQ ID NO: 116 - protein, 17 aa, synthetic construct
DANPNWGGTTHNPRFKG

SEQ ID NO: 117 - protein, 17 aa, synthetic construct
DANPNYGGTTHNPRFKG

SEQ ID NO: 118 - protein, 40 aa, synthetic construct
ARCEPPAVGTACTRLCRPRSAPSRCGPGLRPCAPLEDECE

SEQ ID NO: 119 - protein, 34 aa, synthetic construct
APLVCRAGCSPEHGFCEQPGECRCLEGWTGPLCT

SEQ ID NO: 120 - protein, 37 aa, synthetic construct
GPGPCDGNPCANGGSCSETPRSFECTCPRGFYGLRCE

SEQ ID NO: 121 - protein, 40 aa, synthetic construct
SGVTCADGPCFNGGLCVGGADPDSAYICHCPPGFQGSNCE

SEQ ID NO: 122 - protein, 37 aa, synthetic construct
RVDRCSLQPCRNGGLCLDLGHALRCRCRAGFAGPRCE

SEQ ID NO: 123 - protein, 35 aa, synthetic construct
DDCAGRACANGGTCVEGGGAHRCSCALGFGGRDCR

SEQ ID NO: 124 - protein, 37 aa, synthetic construct
RADPCAARPCAHGGRCYAHFSGLVCACAPGYMGARCE

SEQ ID NO: 125 - protein, 27 aa, synthetic construct
FPVHPDGASALPAAPPGLRPGDPQRYL